European Patent Specification EP 3 807 316 B1, published May 1, 2024. Title: COMPOSITIONS AND METHODS FOR TREATING CANCER. Applicant: INNATE PHARMA. The sequence listing filed with the application follows.

SEQUENCE LISTING (44 sequences)

SEQ ID NO: 1 - protein, 510 aa, Homo sapiens
MEDTKESNVKTFCSKNILAILGFSSIIAVIALLAVGLTQNKALPENVKYGIVLDAGSSHTSLYIYKWPAEKENDTGVVHQVEECRVKGPGISKFVQKVNEIGIYLTDCMERAREVIPRSQHQETPVYLGATAGMRLLRMESEELADRVLDVVERSLSNYPFDFQGARIITGQEEGAYGWITINYLLGKFSQKTRWFSIVPYETNNQETFGALDLGGASTQVTFVPQNQTIESPDNALQFRLYGKDYNVYTHSFLCYGKDQALWQKLAKDIQVASNEILRDPCFHPGYKKVVNVSDLYKTPCTKRFEMTLPFQQFEIQGIGNYQQCHQSILELFNTSYCPYSQCAFNGIFLPPLQGDFGAFSAFYFVMKFLNLTSEKVSQEKVTEMMKKFCAQPWEEIKTSYAGVKEKYLSEYCFSGTYILSLLLQGYHFTADSWEHIHFIGKIQGSDAGWTLGYMLNLTNMIPAEQPLSTPLSHSTYVFLMVLFSLVLFTVAIIGLLIFHKPSYFWKDMV

SEQ ID NO: 2 - protein, 472 aa, Homo sapiens
MAGKVRSLLPPLLLAAAGLAGLLLLCVPTRDVREPPALKYGIVLDAGSSHTSMFIYKWPADKENDTGIVGQHSSCDVPGGGISSYADNPSGASQSLVGCLEQALQDVPKERHAGTPLYLGATAGMRLLNLTNPEASTSVLMAVTHTLTQYPFDFRGARILSGQEEGVFGWVTANYLLENFIKYGWVGRWFRPRKGTLGAMDLGGASTQITFETTSPAEDRASEVQLHLYGQHYRVYTHSFLCYGRDQVLQRLLASALQTHGFHPCWPRGFSTQVLLGDVYQSPCTMAQRPQNFNSSARVSLSGSSDPHLCRDLVSGLFSFSSCPFSRCSFNGVFQPPVAGNFVAFSAFFYTVDFLRTSMGLPVATLQQLEAAAVNVCNQTWAQQLLSRGYGFDERAFGGVIFQKKAADTAVGWALGYMLNLTNLIPADPPGLRKGTDFSSWVVLLLLFASALLAALVLLLRQVHSAKLPSTI

SEQ ID NO: 3 - protein, 484 aa, Homo sapiens
MKKGIRYETSRKTSYIFQQPQHGPWQTRMRKISNHGSLRVAKVAYPLGLCVGVFIYVAYIKWHRATATQAFFSITRAAPGARWGQQAHSPLGTAADGHEVFYGIMFDAGSTGTRVHVFQFTRPPRETPTLTHETFKALKPGLSAYADDVEKSAQGIRELLDVAKQDIPFDFWKATPLVLKATAGLRLLPGEKAQKLLQKVKEVFKASPFLVGDDCVSIMNGTDEGVSAWITINFLTGSLKTPGGSSVGMLDLGGGSTQIAFLPRVEGTLQASPPGYLTALRMFNRTYKLYSYSYLGLGLMSARLAILGGVEGQPAKDGKELVSPCLSPSFKGEWEHAEVTYRVSGQKAAASLHELCAARVSEVLQNRVHRTEEVKHVDFYAFSYYYDLAAGVGLIDAEKGGSLVVGDFEIAAKYVCRTLETQPQSSPFSCMDLTYVSLLLQEFGFPRSKVLKLTRKIDNVETSWALGAIFHYIDSLNRQKSPAS

SEQ ID NO: 4 - protein, 529 aa, Homo sapiens
MFTVLTRQPCEQAGLKALYRTPTIIALVVLLVSIVVLVSITVIQIHKQEVLPPGLKYGIVLDAGSSRTTVYVYQWPAEKENNTGVVSQTFKCSVKGSGISSYGNNPQDVPRAFEECMQKVKGQVPSHLHGSTPIHLGATAGMRLLRLQNETAANEVLESIQSYFKSQPFDFRGAQIISGQEEGVYGWITANYLMGNFLEKNLWHMWVHPHGVETTGALDLGGASTQISFVAGEKMDLNTSDIMQVSLYGYVYTLYTHSFQCYGRNEAEKKFLAMLLQNSPTKNHLTNPCYPRDYSISFTMGHVFDSLCTVDQRPESYNPNDVITFEGTGDPSLCKEKVASIFDFKACHDQETCSFDGVYQPKIKGPFVAFAGFYYTASALNLSGSFSLDTFNSSTWNFCSQNWSQLPLLLPKFDEVYARSYCFSANYIYHLFVNGYKFTEETWPQIHFEKEVGNSSIAWSLGYMLSLTNQIPAESPLIRLPIEPPVFVGTLAFFTAAALLCLAFLAYLCSATRRKRHSEHAFDHAVDSD

SEQ ID NO: 5 - protein, 428 aa, Homo sapiens
MATSWGTVFFMLVVSCVCSAVSHRNQQTWFEGIFLSSMCPINVSASTLYGIMFDAGSTGTRIHVYTFVQKMPGQLPILEGEVFDSVKPGLSAFVDQPKQGAETVQGLLEVAKDSIPRSHWKKTPVVLKATAGLRLLPEHKAKALLFEVKEIFRKSPFLVPKGSVSIMDGSDEGILAWVTVNFLTGQLHGHRQETVGTLDLGGASTQITFLPQFEKTLEQTPRGYLTSFEMFNSTYKLYTHSYLGFGLKAARLATLGALETEGTDGHTFRSACLPRWLEAEWIFGGVKYQYGGNQEGEVGFEPCYAEVLRVVRGKLHQPEEVQRGSFYAFSYYYDRAVDTDMIDYEKGGILKVEDFERKAREVCDNLENFTSGSPFLCMDLSYITALLKDGFGFADSTVLQLTKKVNNIETGWALGATFHLLQSLGISH

SEQ ID NO: 6 - protein, 116 aa, Artificial
  Synthetic
EVQLQQSGPELVKPGASVKMSCKASGYTFTDYNMHWVKQSHGRTLEWIGYIVPLNGGSTFNQKFKGRATLTVNTSSRTAYMELRSLTSEDSAAYYCARGGTRFAYWGQGTLVTVSA

SEQ ID NO: 7 - protein, 111 aa, Artificial
  Synthetic
DIVLTQSPASLAVSLGQRATISCRASESVDNFGVSFMYWFQQKPGQPPNLLIYGASNQGSGVPARFRGSGSGTDFSLNIHPMEADDTAMYFCQQTKEVPYTFGGGTKLEIK

SEQ ID NO: 8 - protein, 5 aa, Mus musculus
DYNMH

SEQ ID NO: 9 - protein, 17 aa, Mus musculus
YIVPLNGGSTFNQKFKG

SEQ ID NO: 10 - protein, 7 aa, Mus musculus
GGTRFAY

SEQ ID NO: 11 - protein, 15 aa, Mus musculus
RASESVDNFGVSFMY

SEQ ID NO: 12 - protein, 7 aa, Mus musculus
GASNQGS

SEQ ID NO: 13 - protein, 9 aa, Mus musculus
QQTKEVPYT

SEQ ID NO: 14 - protein, 17 aa, Artificial
  Synthetic
  X (12)..(12): X may be any amino acid residue
  X (16)..(16): X may be any amino acid residue
YIVPLNGGSTFXQKFXG

SEQ ID NO: 15 - protein, 17 aa, Artificial
  Synthetic
YIVPLNGGSTFSQKFKG

SEQ ID NO: 16 - protein, 17 aa, Artificial
  Synthetic
YIVPLNGGSTFSQKFQG

SEQ ID NO: 17 - protein, 15 aa, Artificial
  Synthetic
  X (1)..(1): X may be any amino acid residue
XASESVDNFGVSFMY

SEQ ID NO: 18 - protein, 15 aa, Artificial
  Synthetic
KASESVDNFGVSFMY

SEQ ID NO: 19 - protein, 218 aa, Artificial
  Synthetic
DIVMTQSPASLAVSLGQRATISCRASESVDNFGVSFMYWFQQKPGQPPNLLIYGASNQGSGVPARFRGSGSGTDFSLNIHPMEADDTAMYFCQQTKEVPYTFGGGTKLEIKRTVAAPSVFIFPPSDEQLKSGTASVVCLLNNFYPREAKVQWKVDNALQSGNSQESVTEQDSKDSTYSLSSTLTLSKADYEKHKVYACEVTHQGLSSPVTKSFNRGEC

SEQ ID NO: 20 - protein, 221 aa, Artificial
  Synthetic
EVKLQQSGPELVKPGASVKMSCKASGYTFTDYNMHWVKQSPGRTLEWIGYIVPLNGGSTFNQKFKGRATLTVNTSSRTAYMELRSLTSEDSAAYYCARGGTRFAYWGQGTLVTVSAASTKGPSVFPLAPSSKSTSGGTAALGCLVKDYFPEPVTVSWNSGALTSGVHTFPAVLQSSGLYSLSSVVTVPSSSLGTQTYICNVNHKPSNTKVDKRVEPKSCDK

SEQ ID NO: 21 - protein, 218 aa, Artificial
  Synthetic
DIVMTQSPDSLAVSLGERATINCRASESVDNFGVSFMYWYQQKPGQPPKLLIYGASNQGSGVPDRFSGSGSGTDFTLTISSLQAEDVAVYYCQQTKEVPYTFGGGTKVEIKRTVAAPSVFIFPPSDEQLKSGTASVVCLLNNFYPREAKVQWKVDNALQSGNSQESVTEQDSKDSTYSLSSTLTLSKADYEKHKVYACEVTHQGLSSPVTKSFNRGEC

SEQ ID NO: 22 - protein, 221 aa, Artificial
  Synthetic
QVQLVQSGAEVKKPGASVKVSCKASGYTFTDYNMHWVRQAPGQRLEWMGYIVPLNGGSTFNQKFKGRVTITRDTSASTAYMELSSLRSEDTAVYYCARGGTRFAYWGQGTLVTVSSASTKGPSVFPLAPSSKSTSGGTAALGCLVKDYFPEPVTVSWNSGALTSGVHTFPAVLQSSGLYSLSSVVTVPSSSLGTQTYICNVNHKPSNTKVDKRVEPKSCDK

SEQ ID NO: 23 - protein, 330 aa, Artificial
  Synthetic
ASTKGPSVFPLAPSSKSTSGGTAALGCLVKDYFPEPVTVSWNSGALTSGVHTFPAVLQSSGLYSLSSVVTVPSSSLGTQTYICNVNHKPSNTKVDKRVEPKSCDKTHTCPPCPAPEAEGGPSVFLFPPKPKDTLMISRTPEVTCVVVDVSHEDPEVKFNWYVDGVEVHNAKTKPREEQYNSTYRVVSVLTVLHQDWLNGKEYKCKVSNKALPASIEKTISKAKGQPREPQVYTLPPSREEMTKNQVSLTCLVKGFYPSDIAVEWESNGQPENNYKTTPPVLDSDGSFFLYSKLTVDKSRWQQGNVFSCSVMHEALHNHYTQKSLSLSPGK

SEQ ID NO: 24 - protein, 330 aa, Artificial
  Synthetic
ASTKGPSVFPLAPSSKSTSGGTAALGCLVKDYFPEPVTVSWNSGALTSGVHTFPAVLQSSGLYSLSSVVTVPSSSLGTQTYICNVNHKPSNTKVDKRVEPKSCDKTHTCPPCPAPEFEGGPSVFLFPPKPKDTLMISRTPEVTCVVVDVSHEDPEVKFNWYVDGVEVHNAKTKPREEQYNSTYRVVSVLTVLHQDWLNGKEYKCKVSNKALPASIEKTISKAKGQPREPQVYTLPPSREEMTKNQVSLTCLVKGFYPSDIAVEWESNGQPENNYKTTPPVLDSDGSFFLYSKLTVDKSRWQQGNVFSCSVMHEALHNHYTQKSLSLSPGK

SEQ ID NO: 25 - protein, 330 aa, Artificial
  Synthetic
ASTKGPSVFPLAPSSKSTSGGTAALGCLVKDYFPEPVTVSWNSGALTSGVHTFPAVLQSSGLYSLSSVVTVPSSSLGTQTYICNVNHKPSNTKVDKRVEPKSCDKTHTCPPCPAPEAEGAPSVFLFPPKPKDTLMISRTPEVTCVVVDVSHEDPEVKFNWYVDGVEVHNAKTKPREEQYNSTYRVVSVLTVLHQDWLNGKEYKCKVSNKALPSSIEKTISKAKGQPREPQVYTLPPSREEMTKNQVSLTCLVKGFYPSDIAVEWESNGQPENNYKTTPPVLDSDGSFFLYSKLTVDKSRWQQGNVFSCSVMHEALHNHYTQKSLSLSPGK

SEQ ID NO: 26 - protein, 330 aa, Artificial
  Synthetic
ASTKGPSVFPLAPSSKSTSGGTAALGCLVKDYFPEPVTVSWNSGALTSGVHTFPAVLQSSGLYSLSSVVTVPSSSLGTQTYICNVNHKPSNTKVDKRVEPKSCDKTHTCPPCPAPEAEGAPSVFLFPPKPKDTLMISRTPEVTCVVVDVSHEDPEVKFNWYVDGVEVHNAKTKPREEQYNSTYRVVSVLTVLHQDWLNGKEYKCKVSNKALPASIEKTISKAKGQPREPQVYTLPPSREEMTKNQVSLTCLVKGFYPSDIAVEWESNGQPENNYKTTPPVLDSDGSFFLYSKLTVDKSRWQQGNVFSCSVMHEALHNHYTQKSLSLSPGK

SEQ ID NO: 27 - protein, 116 aa, Artificial
  Synthetic
QVQLVQSGAEVKKPGASVKVSCKASGYTFTDYNMHWVRQAPGQRLEWMGYIVPLNGGSTFNQKFKGRVTITRDTSASTAYMELSSLRSEDTAVYYCARGGTRFAYWGQGTLVTVSS

SEQ ID NO: 28 - protein, 115 aa, Artificial
  Synthetic
QVQLVQSGAEVKKPGASVKVSCKASGYTFTDYNMHWVRQAPGQRLEWMGYIVPLNGGSTFNQKFKGRVTITVDTSASTAYMELSSLRSEDTAVYYCARGGTRFAYWGQGTLVTVS

SEQ ID NO: 29 - protein, 116 aa, Artificial
  Synthetic
QVQLVQSGAEVKKPGASVKVSCKASGYTFTDYNMHWVRQAPGQRLEWMGYIVPLNGGSTFNQKFKGRATITVDTSASTAYMELSSLRSEDTAVYYCARGGTRFAYWGQGTLVTVSS

SEQ ID NO: 30 - protein, 116 aa, Artificial
  Synthetic
QVQLVQSGAEVKKPGASVKVSCKASGYTFTDYNMHWVRQAPGQRLEWIGYIVPLNGGSTFNQKFKGRATITVDTSASTAYMELSSLRSEDTAVYYCARGGTRFAYWGQGTLVTVSS

SEQ ID NO: 31 - protein, 116 aa, Artificial
  Synthetic
QVQLVQSGAEVKKPGASVKVSCKASGYTFTDYNMHWVRQAPGQRLEWIGYIVPLNGGSTFNQKFKGRATITVDTSARTAYMELSSLRSEDTAVYYCARGGTRFAYWGQGTLVTVSS

SEQ ID NO: 32 - protein, 116 aa, Artificial
  Synthetic
QVQLVQSGAEVKKPGASVKVSCKASGYTFTDYNMHWVRQAPGQRLEWMGYIVPLNGGSTFSQKFKGRATITVDTSASTAYMELSSLRSEDTAVYYCARGGTRFAYWGQGTLVTVSS

SEQ ID NO: 33 - protein, 116 aa, Artificial
  Synthetic
QVQLVQSGAEVKKPGASVKVSCKASGYTFTDYNMHWVRQAPGQRLEWIGYIVPLNGGSTFSQKFQGRATITVDTSASTAYMELSSLRSEDTAVYYCARGGTRFAYWGQGTLVTVSS

SEQ ID NO: 34 - protein, 116 aa, Artificial
  Synthetic
QVQLVQSGAEVKKPGASVKVSCKASGYTFTDYNMHWVRQAPGQRLEWIGYIVPLNGGSTFSQKFQGRATITVDTSARTAYMELSSLRSEDTAVYYCARGGTRFAYWGQGTLVTVSS

SEQ ID NO: 35 - protein, 111 aa, Artificial
  Synthetic
DIVMTQSPDSLAVSLGERATINCRASESVDNFGVSFMYWYQQKPGQPPKLLIYGASNQGSGVPDRFSGSGSGTDFTLTISSLQAEDVAVYYCQQTKEVPYTFGGGTKVEIK

SEQ ID NO: 36 - protein, 111 aa, Artificial
  Synthetic
DIVMTQSPDSLAVSLGERATINCRASESVDNFGVSFMYWFQQKPGQPPKLLIYGASNQGSGVPDRFSGSGSGTDFTLTISSLQAEDVAVYYCQQTKEVPYTFGGGTKVEIK

SEQ ID NO: 37 - protein, 111 aa, Artificial
  Synthetic
DIVMTQSPDSLAVSLGERATINCKASESVDNFGVSFMYWFQQKPGQPPKLLIYGASNQGSGVPDRFSGSGSGTDFTLTISSLQAEDVAVYYCQQTKEVPYTFGGGTKVEIK

SEQ ID NO: 38 - protein, 446 aa, Artificial
  Synthetic
QVQLVQSGAEVKKPGASVKVSCKASGYTFTDYNMHWVRQAPGQRLEWIGYIVPLNGGSTFNQKFKGRATITVDTSARTAYMELSSLRSEDTAVYYCARGGTRFAYWGQGTLVTVSSASTKGPSVFPLAPSSKSTSGGTAALGCLVKDYFPEPVTVSWNSGALTSGVHTFPAVLQSSGLYSLSSVVTVPSSSLGTQTYICNVNHKPSNTKVDKRVEPKSCDKTHTCPPCPAPEAEGAPSVFLFPPKPKDTLMISRTPEVTCVVVDVSHEDPEVKFNWYVDGVEVHNAKTKPREEQYNSTYRVVSVLTVLHQDWLNGKEYKCKVSNKALPSSIEKTISKAKGQPREPQVYTLPPSREEMTKNQVSLTCLVKGFYPSDIAVEWESNGQPENNYKTTPPVLDSDGSFFLYSKLTVDKSRWQQGNVFSCSVMHEALHNHYTQKSLSLSPGK

SEQ ID NO: 39 - protein, 218 aa, Artificial
  Synthetic
DIVMTQSPDSLAVSLGERATINCRASESVDNFGVSFMYWFQQKPGQPPKLLIYGASNQGSGVPDRFSGSGSGTDFTLTISSLQAEDVAVYYCQQTKEVPYTFGGGTKVEIKRTVAAPSVFIFPPSDEQLKSGTASVVCLLNNFYPREAKVQWKVDNALQSGNSQESVTEQDSKDSTYSLSSTLTLSKADYEKHKVYACEVTHQGLSSPVTKSFNRGEC

SEQ ID NO: 40 - protein, 218 aa, Artificial
  Synthetic
DIVMTQSPDSLAVSLGERATINCKASESVDNFGVSFMYWFQQKPGQPPKLLIYGASNQGSGVPDRFSGSGSGTDFTLTISSLQAEDVAVYYCQQTKEVPYTFGGGTKVEIKRTVAAPSVFIFPPSDEQLKSGTASVVCLLNNFYPREAKVQWKVDNALQSGNSQESVTEQDSKDSTYSLSSTLTLSKADYEKHKVYACEVTHQGLSSPVTKSFNRGEC

SEQ ID NO: 41 - DNA, 45 bp, Homo sapiens
tacgactcacaagcttgccgccaccatggaagatacaaaggagtc

SEQ ID NO: 42 - DNA, 64 bp, Homo sapiens
ccgccccgactctagatcacttgtcatcgtcatctttgtaatcgacataggtggagtgggagag

SEQ ID NO: 43 - protein, 478 aa, homo sapiens
MEDTKESNVKTFCSKNILAILGFSSIIAVIALLAVGLTQNKALPENVKYGIVLDAGSSHTSLYIYKWPAEKENDTGVVHQVEECRVKGPGISKFVQKVNEIGIYLTDCMERAREVIPRSQHQETPVYLGATAGMRLLRMESEELADRVLDVVERSLSNYPFDFQGARIITGQEEGAYGWITINYLLGKFSQKTRWFSIVPYETNNQETFGALDLGGASTQVTFVPQNQTIESPDNALQFRLYGKDYNVYTHSFLCYGKDQALWQKLAKDIQVASNEILRDPCFHPGYKKVVNVSDLYKTPCTKRFEMTLPFQQFEIQGIGNYQQCHQSILELFNTSYCPYSQCAFNGIFLPPLQGDFGAFSAFYFVMKFLNLTSEKVSQEKVTEMMKKFCAQPWEEIKTSYAGVKEKYLSEYCFSGTYILSLLLQGYHFTADSWEHIHFIGKIQGSDAGWTLGYMLNLTNMIPAEQPLSTPLSHSTYV

SEQ ID NO: 44 - protein, 486 aa, Artificial
  Synthetic
MEDTKESNVKTFCSKNILAILGFSSIIAVIALLAVGLTQNKALPENVKYGIVLDAGSSHTSLYIYKWPAEKENDTGVVHQVEECRVKGPGISKFVQKVNEIGIYLTDCMERAREVIPRSQHQETPVYLGATAGMRLLRMESEELADRVLDVVERSLSNYPFDFQGARIITGQEEGAYGWITINYLLGKFSQKTRWFSIVPYETNNQETFGALDLGGASTQVTFVPQNQTIESPDNALQFRLYGKDYNVYTHSFLCYGKDQALWQKLAKDIQVASNEILRDPCFHPGYKKVVNVSDLYKTPCTKRFEMTLPFQQFEIQGIGNYQQCHQSILELFNTSYCPYSQCAFNGIFLPPLQGDFGAFSAFYFVMKFLNLTSEKVSQEKVTEMMKKFCAQPWEEIKTSYAGVKEKYLSEYCFSGTYILSLLLQGYHFTADSWEHIHFIGKIQGSDAGWTLGYMLNLTNMIPAEQPLSTPLSHSTYVDYKDDDDK